European Patent Specification EP 3 728 328 B1, published October 23, 2024. Title: BISPECIFIC ANTIGEN BINDING CONSTRUCT. Applicant: ARGENX BVBA. The sequence listing filed with the application follows.

SEQUENCE LISTING (36 sequences)

SEQ ID NO: 1 - protein, 10 aa, Homo sapiens
EPKSCDKTHT

SEQ ID NO: 2 - protein, 5 aa, Homo sapiens
CPPCP

SEQ ID NO: 3 - protein, 8 aa, Homo sapiens
APELLGGP

SEQ ID NO: 4 - protein, 10 aa, Homo sapiens
CCVECPPPCP

SEQ ID NO: 5 - protein, 7 aa, Homo sapiens
APPVAGP

SEQ ID NO: 6 - protein, 12 aa, Homo sapiens
ELKTPLGDTTHT

SEQ ID NO: 7 - protein, 50 aa, Homo sapiens
CPRCPEPKSCDTPPPCPRCPEPKSCDTPPPCPRCPEPKSCDTPPPCPRCP

SEQ ID NO: 8 - protein, 7 aa, Homo sapiens
ESKYGPP

SEQ ID NO: 9 - protein, 5 aa, Homo sapiens
CPSCP

SEQ ID NO: 10 - protein, 8 aa, Homo sapiens
APEFLGGP

SEQ ID NO: 11 - DNA, 373 bp, Artificial sequence
  Synthetic polynucleotide
gagttgcaggtggtggagtctgggggaggattggtgcaggctggggcctctctgagactctcctgtgtagcctctggacgcaccttcagtagttattccatggcctggttccgccaggctccagggaaggagcgtgagtttgtcgcgacggttagtaattggaatgattacatcacaacctatgcagactccgtgaagggccgattcaccatctccagagacaatgccaaaaacacggtgtctctgcaaatgaacggcctgaaacctgaggacacggccgtttattactgtgcagcgcggaccggggctcctagggtcacttccggacagtatgactactggggccaggggacccaggtcaccgtgtcctcag

SEQ ID NO: 12 - protein, 124 aa, Artificial sequence
  Synthetic polypeptide
ELQVVESGGGLVQAGASLRLSCVASGRTFSSYSMAWFRQAPGKEREFVATVSNWNDYITTYADSVKGRFTISRDNAKNTVSLQMNGLKPEDTAVYYCAARTGAPRVTSGQYDYWGQGTQVTVSS

SEQ ID NO: 13 - DNA, 361 bp, Artificial sequence
  Synthetic polynucleotide
gagttgcagctggtggagtctgggggaggcttggtgcagcctggggggtctcggagactctcctgtgctgcctctgggttcacctacagtgactactggatgtattgggtccgtcagcctccagggaagggactcgagtgggtctcaaatattaattctgaaggtggtagcacagcctatgcagactccgtgaagggccgattcaccatctccagagacaacgccaagaacacgctgtatctgcaaatgaacagtctgaaatctgaggacacggccgtatactactgtgtaagagcattaagcagtggtcaatggtacccggcctactggggccaggggacccaggtcaccgtgtcctccg

SEQ ID NO: 14 - protein, 120 aa, Artificial sequence
  Synthetic polypeptide
ELQLVESGGGLVQPGGSRRLSCAASGFTYSDYWMYWVRQPPGKGLEWVSNINSEGGSTAYADSVKGRFTISRDNAKNTLYLQMNSLKSEDTAVYYCVRALSSGQWYPAYWGQGTQVTVSS

SEQ ID NO: 15 - DNA, 796 bp, Artificial sequence
  Synthetic polynucleotide
ctgtcgtctcactctgagttgcagctggtggagtctgggggaggcttggtgcagcctggggggtctcggagactctcctgtgctgcctctgggttcacctacagtgactactggatgtattgggtccgtcagcctccagggaagggactcgagtgggtctcaaatattaattctgaaggtggtagcacagcctatgcagactccgtgaagggccgattcaccatctccagagacaacgccaagaacacgctgtatctgcaaatgaacagtctgaaatctgaggacacggccgtatactactgtgtaagagcattaagcagtggtcaatggtacccggcctactggggccaggggacccaggtcaccgtgtcctccgcctccgcggccgcaagcggtggaggcggttcaggcggaggtggatctggcggtggcggaagtgcacaggcagggctgactcagctgccctccgtgtctggatccccaggccagaagatcaccatctcctgcactggaagcagcagcaacatcagggttggttataatgttcagcggttccagcacctcccaggaacacccccccaactgctcatctatggtaacagcaatcaagcttcgggggtcccagaccgcttctctggctccaagtctggcagctcggcctccctgaccatcactgggctccaggctgaggacgaggctgactattactgtgaatgctatgacagcggcctcagtgggcctgtgttcggcggagggaccaagctgaccgtcctcggtgagcctgagacgacacgcc

SEQ ID NO: 16 - protein, 260 aa, Artificial sequence
  Synthetic polypeptide
ELQLVESGGGLVQPGGSRRLSCAASGFTYSDYWMYWVRQPPGKGLEWVSNINSEGGSTAYADSVKGRFTISRDNAKNTLYLQMNSLKSEDTAVYYCVRALSSGQWYPAYWGQGTQVTVSSASAAASGGGGSGGGGSGGGGSAQAGLTQLPSVSGSPGQKITISCTGSSSNIRVGYNVQRFQHLPGTPPQLLIYGNSNQASGVPDRFSGSKSGSSASLTITGLQAEDEADYYCECYDSGLSGPVFGGGTKLTVLGEPETTR

SEQ ID NO: 17 - DNA, 1104 bp, Artificial sequence
  Synthetic polynucleotide
cgtttaaacggtaccgccgccaccatgggctggtcctgcatcatcctgtttctggtggccaccgccacaggcgtccactctggagacgccaatccttcactcgaattccgtctcgctaaaacaacagccccatcggtctatccactggcccctgtgtgtggagatacaactggctcctcggtgactctaggatgcctggtcaagggttatttccctgagccagtgaccttgacctggaactctggatccctgtccagtggtgtgcacaccttcccagctgtcctgcagtctgacctctacaccctcagcagctcagtgactgtaacctcgagcacctggcccagccagtccatcacctgcaatgtggcccacccggcaagcagcaccaaggtggacaagaaaattgagcccagagggcccacaatcaagccctgtcctccatgcaaatgcccagcacctaacctcttgggtggaccagacgtcttcatcttccctccaaagatcaaggatgtactcatgatctccctgagccccatagtcacatgtgtggtggtggatgtgagcgaggatgacccagatgtccagatcagctggtttgtgaacaacgtggaagtacacacagctcagacacaaacccatagagaggattaccagagtactctccgggtggtcagtgccctccccatccagcaccaggactggatgagtggcaaggagttcaaatgcaaggtcaacaacaaagacctcccagcgcccgaagagagaaccatctcaaaacccaaagggtcagtaagagctccacaggtatatgtcttgcctccaccagaagaagagatgactaagaaacaggtcactctgtcctgcgctgtcacagacttcatgcctgaagacatttacgtggagtggaccaacaacgggaaaacagagctaaactacaagaacactgaaccagtcctggactctgatggttcttacttcatggtgagcaagctgagagtggaaaagaagaactgggtggaaagaaatagctactcctgttcagtggtccacgagggtctgcacaatcaccacacgactaagagcttctcccggactccgggtaaa

SEQ ID NO: 18 - protein, 368 aa, Artificial sequence
  Synthetic polypeptide
RLNGTAATMGWSCIILFLVATATGVHSGDANPSLEFRLAKTTAPSVYPLAPVCGDTTGSSVTLGCLVKGYFPEPVTLTWNSGSLSSGVHTFPAVLQSDLYTLSSSVTVTSSTWPSQSITCNVAHPASSTKVDKKIEPRGPTIKPCPPCKCPAPNLLGGPDVFIFPPKIKDVLMISLSPIVTCVVVDVSEDDPDVQISWFVNNVEVHTAQTQTHREDYQSTLRVVSALPIQHQDWMSGKEFKCKVNNKDLPAPEERTISKPKGSVRAPQVYVLPPPEEEMTKKQVTLSCAVTDFMPEDIYVEWTNNGKTELNYKNTEPVLDSDGSYFMVSKLRVEKKNWVERNSYSCSVVHEGLHNHHTTKSFSRTPGK

SEQ ID NO: 19 - DNA, 1104 bp, Artificial sequence
  Synthetic polynucleotide
cgtttaaacggtaccgccgccaccatgggctggtcctgcatcatcctgtttctggtggccaccgccacaggcgtccactctggagacgccaatccttcactcgaattccgtctcgctaaaacaacagccccatcggtctatccactggcccctgtgtgtggagatacaactggctcctcggtgactctaggatgcctggtcaagggttatttccctgagccagtgaccttgacctggaactctggatccctgtccagtggtgtgcacaccttcccagctgtcctgcagtctgacctctacaccctcagcagctcagtgactgtaacctcgagcacctggcccagccagtccatcacctgcaatgtggcccacccggcaagcagcaccaaggtggacaagaaaattgagcccagagggcccacaatcaagccctgtcctccatgcaaatgcccagcacctaacctcttgggtggaccagacgtcttcatcttccctccaaagatcaaggatgtactcatgatctccctgagccccatagtcacatgtgtggtggtggatgtgagcgaggatgacccagatgtccagatcagctggtttgtgaacaacgtggaagtacacacagctcagacacaaacccatagagaggattacaacagtactctccgggtggtcagtgccctccccatccagcaccaggactggatgagtggcaaggagttcaaatgcaaggtcaacaacaaagacctcccagcgcccgaagagagaaccatctcaaaacccaaagggtcagtaagagctccacaggtatatgtcttgcctccaccagaagaagagatgactaagaaacaggtcactctgtggtgcatggtcacagacttcatgcctgaagacatttacgtggagtggaccaacaacgggaaaacagagctaaactacaagaacactgaaccagtcctggactctgatggttcttacttcatgtacagcaagctgagagtggaaaagaagaactgggtggaaagaaatagctactcctgttcagtggtccacgagggtctgcacaatcaccacacgactaagagcttctcccggactccgggtaaa

SEQ ID NO: 20 - protein, 368 aa, Artificial sequence
  Synthetic polypeptide
RLNGTAATMGWSCIILFLVATATGVHSGDANPSLEFRLAKTTAPSVYPLAPVCGDTTGSSVTLGCLVKGYFPEPVTLTWNSGSLSSGVHTFPAVLQSDLYTLSSSVTVTSSTWPSQSITCNVAHPASSTKVDKKIEPRGPTIKPCPPCKCPAPNLLGGPDVFIFPPKIKDVLMISLSPIVTCVVVDVSEDDPDVQISWFVNNVEVHTAQTQTHREDYNSTLRVVSALPIQHQDWMSGKEFKCKVNNKDLPAPEERTISKPKGSVRAPQVYVLPPPEEEMTKKQVTLWCMVTDFMPEDIYVEWTNNGKTELNYKNTEPVLDSDGSYFMYSKLRVEKKNWVERNSYSCSVVHEGLHNHHTTKSFSRTPGK

SEQ ID NO: 21 - DNA, 813 bp, Artificial sequence
  Synthetic polynucleotide
cgtttaaacggtaccgccgccaccatgggctggtcctgcatcatcctgtttctggtggccaccgccacaggcgtccactctggagacgccaatccttcactcgaattccgtctcgagcccagagggcccacaatcaagccctgtcctccatgcaaatgcccagcacctaacctcttgggtggaccagacgtcttcatcttccctccaaagatcaaggatgtactcatgatctccctgagccccatagtcacatgtgtggtggtggatgtgagcgaggatgacccagatgtccagatcagctggtttgtgaacaacgtggaagtacacacagctcagacacaaacccatagagaggattacaacagtactctccgggtggtcagtgccctccccatccagcaccaggactggatgagtggcaaggagttcaaatgcaaggtcaacaacaaagacctcccagcgcccgaagagagaaccatctcaaaacccaaagggtcagtaagagctccacaggtatatgtcttgcctccaccagaagaagagatgactaagaaacaggtcactctgtcctgcgctgtcacagacttcatgcctgaagacatttacgtggagtggaccaacaacgggaaaacagagctaaactacaagaacactgaaccagtcctggactctgatggttcttacttcatggtgagcaagctgagagtggaaaagaagaactgggtggaaagaaatagctactcctgttcagtggtccacgagggtctgcacaatcaccacacgactaagagcttctcccggactccgggtaaa

SEQ ID NO: 22 - protein, 271 aa, Artificial sequence
  Synthetic polypeptide
RLNGTAATMGWSCIILFLVATATGVHSGDANPSLEFRLEPRGPTIKPCPPCKCPAPNLLGGPDVFIFPPKIKDVLMISLSPIVTCVVVDVSEDDPDVQISWFVNNVEVHTAQTQTHREDYNSTLRVVSALPIQHQDWMSGKEFKCKVNNKDLPAPEERTISKPKGSVRAPQVYVLPPPEEEMTKKQVTLSCAVTDFMPEDIYVEWTNNGKTELNYKNTEPVLDSDGSYFMVSKLRVEKKNWVERNSYSCSVVHEGLHNHHTTKSFSRTPGK

SEQ ID NO: 23 - DNA, 813 bp, Artificial sequence
  Synthetic polynucleotide
cgtttaaacggtaccgccgccaccatgggctggtcctgcatcatcctgtttctggtggccaccgccacaggcgtccactctggagacgccaatccttcactcgaattccgtctcgagcccagagggcccacaatcaagccctgtcctccatgcaaatgcccagcacctaacctcttgggtggaccagacgtcttcatcttccctccaaagatcaaggatgtactcatgatctccctgagccccatagtcacatgtgtggtggtggatgtgagcgaggatgacccagatgtccagatcagctggtttgtgaacaacgtggaagtacacacagctcagacacaaacccatagagaggattacaacagtactctccgggtggtcagtgccctccccatccagcaccaggactggatgagtggcaaggagttcaaatgcaaggtcaacaacaaagacctcccagcgcccgaagagagaaccatctcaaaacccaaagggtcagtaagagctccacaggtatatgtcttgcctccaccagaagaagagatgactaagaaacaggtcactctgtggtgcatggtcacagacttcatgcctgaagacatttacgtggagtggaccaacaacgggaaaacagagctaaactacaagaacactgaaccagtcctggactctgatggttcttacttcatgtacagcaagctgagagtggaaaagaagaactgggtggaaagaaatagctactcctgttcagtggtccacgagggtctgcacaatcaccacacgactaagagcttctcccggactccgggtaaa

SEQ ID NO: 24 - protein, 271 aa, Artificial sequence
  Synthetic polypeptide
RLNGTAATMGWSCIILFLVATATGVHSGDANPSLEFRLEPRGPTIKPCPPCKCPAPNLLGGPDVFIFPPKIKDVLMISLSPIVTCVVVDVSEDDPDVQISWFVNNVEVHTAQTQTHREDYNSTLRVVSALPIQHQDWMSGKEFKCKVNNKDLPAPEERTISKPKGSVRAPQVYVLPPPEEEMTKKQVTLWCMVTDFMPEDIYVEWTNNGKTELNYKNTEPVLDSDGSYFMYSKLRVEKKNWVERNSYSCSVVHEGLHNHHTTKSFSRTPGK

SEQ ID NO: 25 - DNA, 991 bp, Artificial sequence
  Synthetic polynucleotide
agtttaaacggtaccgccgccaccatgggctggtcctgcatcatcctgtttctggtggccaccgccacaggcgtccactctggagacgcctccttaacactcgaattccgtctcgctaaaacaacagccccatcggtctatccactggcccctgtgtgtggagatacaactggctcctcggtgactctaggatgcctggtcaagggttatttccctgagccagtgaccttgacctggaactctggatccctgtccagtggtgtgcacaccttcccagctgtcctgcagtctgacctctacaccctcagcagctcagtgactgtaacctcgagcacctggcccagccagtccatcacctgcaatgtggcccacccggcaagcagcaccaaggtggacaagaaaattgagcccagagggcccacaatcaagccctgtcctccatgcaaatgcccagcacctaacctcttgggtggaccatccgtcttcatcttccctccaaagatcaaggatgtactcatgatctccctgagccccatagtcacatgtgtggtggtggatgtgagcgaggatgacccagatgtccagatcagctggtttgtgaacaacgtggaagtacacacagctcagacacaaacccatagagaggattacaacagtactctccgggtggtcagtgccctccccatccagcaccaggactggatgagtggcaaggagttcaaatgcaaggtcaacaacaaagacctcccagcgcccatcgagagaaccatctcaaaacccaaagggtcagtaagagctccacaggtatatgtcttgcctccaccagaagaagagatgactaagaaacaggtcactctgacctgcatggtcacagacttcatgcctgaagacatttacgtggagtggaccaacaacgggaaaacagagctaaactacaagaacactgaaccagtcctggactctgatggttcttacttcatgtacagcaagc

SEQ ID NO: 26 - protein, 330 aa, Artificial sequence
  Synthetic polypeptide
SLNGTAATMGWSCIILFLVATATGVHSGDASLTLEFRLAKTTAPSVYPLAPVCGDTTGSSVTLGCLVKGYFPEPVTLTWNSGSLSSGVHTFPAVLQSDLYTLSSSVTVTSSTWPSQSITCNVAHPASSTKVDKKIEPRGPTIKPCPPCKCPAPNLLGGPSVFIFPPKIKDVLMISLSPIVTCVVVDVSEDDPDVQISWFVNNVEVHTAQTQTHREDYNSTLRVVSALPIQHQDWMSGKEFKCKVNNKDLPAPIERTISKPKGSVRAPQVYVLPPPEEEMTKKQVTLTCMVTDFMPEDIYVEWTNNGKTELNYKNTEPVLDSDGSYFMYSK

SEQ ID NO: 27 - protein, 330 aa, Artificial sequence
  Synthetic polypeptide
AKTTAPSVYPLAPVCGDTTGSSVTLGCLVKGYFPEPVTLTWNSGSLSSGVHTFPAVLQSDLYTLSSSVTVTSSTWPSQSITCNVAHPASSTKVDKKIEPRGPTIKPCPPCKCPAPNLLGGPDVFIFPPKIKDVLMISLSPIVTCVVVDVSEDDPDVQISWFVNNVEVHTAQTQTHREDYQSTLRVVSALPIQHQDWMSGKEFKCKVNNKDLPAPEERTISKPKGSVRAPQVYVLPPPEEEMTKKQVTLSCAVTDFMPEDIYVEWTNNGKTELNYKNTEPVLDSDGSYFMVSKLRVEKKNWVERNSYSCSVVHEGLHNHHTTKSFSRTPGK

SEQ ID NO: 28 - protein, 233 aa, Artificial sequence
  Synthetic polypeptide
EPRGPTIKPCPPCKCPAPNLLGGPDVFIFPPKIKDVLMISLSPIVTCVVVDVSEDDPDVQISWFVNNVEVHTAQTQTHREDYNSTLRVVSALPIQHQDWMSGKEFKCKVNNKDLPAPEERTISKPKGSVRAPQVYVLPPPEEEMTKKQVTLWCMVTDFMPEDIYVEWTNNGKTELNYKNTEPVLDSDGSYFMYSKLRVEKKNWVERNSYSCSVVHEGLHNHHTTKSFSRTPGK

SEQ ID NO: 29 - protein, 242 aa, Artificial sequence
  Synthetic polypeptide
GGGGSGGGGSEPRGPTIKPCPPCKCPAPNLLGGPSVFIFPPKIKDVLMISLSPIVTCVVVDVSEDDPDVQISWFVNNVEVHTAQTQTHREDYASTLRVVSALPIQHQDWMSGKEFKCKVNNKDLPAPIERTISKPKGSVRAPQVYVLPPPEEEMTKKQVTLWCMVTDFMPEDIYVEWTNNGKTELNYKNTEPVLDSDGSYFMYSKLRVEKKNWVERNSYSCSVVHEGLHNHHTTKSFSRTPG

SEQ ID NO: 30 - protein, 242 aa, Artificial sequence; identical to SEQ ID NO: 29
  Synthetic polypeptide

SEQ ID NO: 31 - protein, 330 aa, Artificial sequence
  Synthetic polypeptide
AKTTAPSVYPLAPVCGDTTGSSVTLGCLVKGYFPEPVTLTWNSGSLSSGVHTFPAVLQSDLYTLSSSVTVTSSTWPSQSITCNVAHPASSTKVDKKIEPRGPTIKPCPPCKCPAPNLLGGPSVFIFPPKIKDVLMISLSPIVTCVVVDVSEDDPDVQISWFVNNVEVHTAQTQTHREDYASTLRVVSALPIQHQDWMSGKEFKCKVNNKDLPAPIERTISKPKGSVRAPQVYVLPPPEEEMTKKQVTLSCAVTDFMPEDIYVEWTNNGKTELNYKNTEPVLDSDGSYFMVSKLRVEKKNWVERNSYSCSVVHEGLHNHHTTKSFSRTPGK

SEQ ID NO: 32 - protein, 373 aa, Artificial sequence
  Synthetic polypeptide
RLNGTAATMGWSCIILFLVATATGVHSGDANPSLEFRLAKTTAPSVYPLAPVCGDTTGSSVTLGCLVKGYFPEPVTLTWNSGSLSSGVHTFPAVLQSDLYTLSSSVTVTSSTWPSQSITCNVAHPASSTKVDKKIEPRGPTIKPCPPCKCPAPNLLGGPDVFIFPPKIKDVLMISLSPIVTCVVVDVSEDDPDVQISWFVNNVEVHTAQTQTHREDYQSTLRVVSALPIQHQDWMSGKEFKCKVNNKDLPAPEERTISKPKGSVRAPQVYVLPPPEEEMTKKQVTLSCAVTDFMPEDIYVEWTNNGKTELNYKNTEPVLDSDGSYFMVSKLRVEKKNWVERNSYSCSVVHEGLHNHHTTKSFSRTPGKSRAAA

SEQ ID NO: 33 - protein, 373 aa, Artificial sequence
  Synthetic polypeptide
RLNGTAATMGWSCIILFLVATATGVHSGDANPSLEFRLAKTTAPSVYPLAPVCGDTTGSSVTLGCLVKGYFPEPVTLTWNSGSLSSGVHTFPAVLQSDLYTLSSSVTVTSSTWPSQSITCNVAHPASSTKVDKKIEPRGPTIKPCPPCKCPAPNLLGGPDVFIFPPKIKDVLMISLSPIVTCVVVDVSEDDPDVQISWFVNNVEVHTAQTQTHREDYNSTLRVVSALPIQHQDWMSGKEFKCKVNNKDLPAPEERTISKPKGSVRAPQVYVLPPPEEEMTKKQVTLWCMVTDFMPEDIYVEWTNNGKTELNYKNTEPVLDSDGSYFMYSKLRVEKKNWVERNSYSCSVVHEGLHNHHTTKSFSRTPGKSRAAA

SEQ ID NO: 34 - protein, 276 aa, Artificial sequence
  Synthetic polypeptide
RLNGTAATMGWSCIILFLVATATGVHSGDANPSLEFRLEPRGPTIKPCPPCKCPAPNLLGGPDVFIFPPKIKDVLMISLSPIVTCVVVDVSEDDPDVQISWFVNNVEVHTAQTQTHREDYNSTLRVVSALPIQHQDWMSGKEFKCKVNNKDLPAPEERTISKPKGSVRAPQVYVLPPPEEEMTKKQVTLSCAVTDFMPEDIYVEWTNNGKTELNYKNTEPVLDSDGSYFMVSKLRVEKKNWVERNSYSCSVVHEGLHNHHTTKSFSRTPGKSRAAA

SEQ ID NO: 35 - protein, 276 aa, Artificial sequence
  Synthetic polypeptide
RLNGTAATMGWSCIILFLVATATGVHSGDANPSLEFRLEPRGPTIKPCPPCKCPAPNLLGGPDVFIFPPKIKDVLMISLSPIVTCVVVDVSEDDPDVQISWFVNNVEVHTAQTQTHREDYNSTLRVVSALPIQHQDWMSGKEFKCKVNNKDLPAPEERTISKPKGSVRAPQVYVLPPPEEEMTKKQVTLWCMVTDFMPEDIYVEWTNNGKTELNYKNTEPVLDSDGSYFMYSKLRVEKKNWVERNSYSCSVVHEGLHNHHTTKSFSRTPGKSRAAA

SEQ ID NO: 36 - protein, 330 aa, Artificial sequence; identical to SEQ ID NO: 26
  Synthetic polypeptide